European Patent Specification EP 3 463 422 B1, published May 22, 2024. Title: COMPOSITIONS AND METHODS FOR TREATING METABOLIC DISEASES. Applicant: SHANGHAI HEP PHARMACEUTICAL CO., LTD. The sequence listing filed with the application follows.

SEQUENCE LISTING (49 sequences)

SEQ ID NO: 1 - protein, 60 aa, Artificial Sequence
  Description of Artificial Sequence: Synthetic polypeptide
  N-term Myr
  C-term NH2
GTNLSVPNPLGFFPDHQLDPAFGANSNNPDWDFNPNKDHWPEANQVGAGAFGPGFTPPHG

SEQ ID NO: 2 - protein, 55 aa, Artificial Sequence
  Description of Artificial Sequence: Synthetic polypeptide
  N-term Myr
  C-term NH2
GTNLSVPNPLGFFPDHQLDPAFGANSNNPDWDFNPNKDHWPEANQVGAGAFGPGF

SEQ ID NO: 3 - protein, 47 aa, Artificial Sequence
  Description of Artificial Sequence: Synthetic polypeptide
  N-term Myr
  C-term NH2
GTNLSVPNPLGFFPDHQLDPAFGANSNNPDWDFNPNKDHWPEANQVG

SEQ ID NO: 4 - protein, 40 aa, Artificial Sequence
  Description of Artificial Sequence: Synthetic polypeptide
  N-term Myr
  C-term NH2
GTNLSVPNPLGFFPDHQLDPAFGANSNNPDWDFNPNKDHW

SEQ ID NO: 5 - protein, 35 aa, Artificial Sequence
  Description of Artificial Sequence: Synthetic polypeptide
  N-term Myr
  C-term NH2
GTNLSVPNPLGFFPDHQLDPAFGANSNNPDWDFNP

SEQ ID NO: 6 - protein, 30 aa, Artificial Sequence
  Description of Artificial Sequence: Synthetic polypeptide
  N-term Myr
  C-term NH2
GTNLSVPNPLGFFPDHQLDPAFGANSNNPD

SEQ ID NO: 7 - protein, 25 aa, Artificial Sequence
  Description of Artificial Sequence: Synthetic peptide
  N-term Myr
  C-term NH2
GTNLSVPNPLGFFPDHQLDPAFGAN

SEQ ID NO: 8 - protein, 20 aa, Artificial Sequence
  Description of Artificial Sequence: Synthetic peptide
  N-term Myr
  C-term NH2
GTNLSVPNPLGFFPDHQLDP

SEQ ID NO: 9 - protein, 58 aa, Artificial Sequence
  Description of Artificial Sequence: Synthetic polypeptide
  N-term Myr
  C-term NH2
GGWSSKPRQGMGTNLSVPNPLGFFPDHQLDPAFGANSNNPDWDFNPNKDHWPEANQVG

SEQ ID NO: 10 - protein, 57 aa, Artificial Sequence
  Description of Artificial Sequence: Synthetic polypeptide
  N-term Myr
  C-term NH2
GLSWTVPLEWGTNLSVPNPLGFFPDHQLDPAFGANSNNPDWDFNPNKDHWPEANQVG

SEQ ID NO: 11 - protein, 47 aa, Artificial Sequence; identical to SEQ ID NO: 3
  Description of Artificial Sequence: Synthetic polypeptide
  N-term Plam
  C-term NH2

SEQ ID NO: 12 - protein, 47 aa, Artificial Sequence; identical to SEQ ID NO: 3
  Description of Artificial Sequence: Synthetic polypeptide
  N-term Stearoyl
  C-term NH2

SEQ ID NO: 13 - protein, 47 aa, Artificial Sequence; identical to SEQ ID NO: 3
  Description of Artificial Sequence: Synthetic polypeptide
  N-term Chol
  C-term NH2

SEQ ID NO: 14 - protein, 47 aa, Artificial Sequence
  Description of Artificial Sequence: Synthetic polypeptide
  N-term Myr
  C-term NH2
GTNLSVPNPLGFFPDHQLDPAFGANSNNPDWDFNPVKDDWPAANQVG

SEQ ID NO: 15 - protein, 47 aa, Artificial Sequence
  Description of Artificial Sequence: Synthetic polypeptide
  N-term Myr
  C-term NH2
GTNLSVPNPLGFFPDHQLDPAFKANSENPDWDLNPNKDNWPDANKVG

SEQ ID NO: 16 - protein, 47 aa, Artificial Sequence
  Description of Artificial Sequence: Synthetic polypeptide
  N-term Myr
  C-term NH2
GQNLSTSNPLGFFPDHQLDPAFRANTANPDWDFNPNKDTWPDANKVG

SEQ ID NO: 17 - protein, 47 aa, Artificial Sequence
  Description of Artificial Sequence: Synthetic polypeptide
  N-term Myr
  C-term NH2
GKNISTTNPLGFFPDHQLDPAFRANTRNPDWDHNPNKDHWTEANKVG

SEQ ID NO: 18 - protein, 47 aa, Artificial Sequence
  Description of Artificial Sequence: Synthetic polypeptide
  N-term Myr
  C-term NH2
GQNLSVPNPLGFFPDHQLDPLFRANSSSPDWDFNTNKDSWPMANKVG

SEQ ID NO: 19 - protein, 47 aa, Artificial Sequence
  Description of Artificial Sequence: Synthetic polypeptide
  N-term Myr
  C-term NH2
GKNLSASNPLGFLPDHQLDPAFRANTNNPDWDFNPKKDPWPEANKVG

SEQ ID NO: 20 - protein, 47 aa, Artificial Sequence
  Description of Artificial Sequence: Synthetic polypeptide
  N-term Myr
  C-term NH2
GQNLSVPNPLGFFPDHQLDPLFRANSSSPDWDFNTNKDNWPMANKVG

SEQ ID NO: 21 - protein, 60 aa, Hepatitis B virus; identical to SEQ ID NO: 1

SEQ ID NO: 22 - protein, 55 aa, Hepatitis B virus; identical to SEQ ID NO: 2

SEQ ID NO: 23 - protein, 47 aa, Hepatitis B virus; identical to SEQ ID NO: 3

SEQ ID NO: 24 - protein, 40 aa, Hepatitis B virus; identical to SEQ ID NO: 4

SEQ ID NO: 25 - protein, 35 aa, Hepatitis B virus; identical to SEQ ID NO: 5

SEQ ID NO: 26 - protein, 30 aa, Hepatitis B virus; identical to SEQ ID NO: 6

SEQ ID NO: 27 - protein, 25 aa, Hepatitis B virus
GTNLSVPNPLGFFPDHQLDPAFGAN

SEQ ID NO: 28 - protein, 20 aa, Hepatitis B virus
GTNLSVPNPLGFFPDHQLDP

SEQ ID NO: 29 - protein, 58 aa, Hepatitis B virus; identical to SEQ ID NO: 9

SEQ ID NO: 30 - protein, 57 aa, Hepatitis B virus; identical to SEQ ID NO: 10

SEQ ID NO: 31 - protein, 47 aa, Hepatitis B virus; identical to SEQ ID NO: 3

SEQ ID NO: 32 - protein, 47 aa, Hepatitis B virus; identical to SEQ ID NO: 3

SEQ ID NO: 33 - protein, 47 aa, Hepatitis B virus; identical to SEQ ID NO: 3

SEQ ID NO: 34 - protein, 47 aa, Hepatitis B virus; identical to SEQ ID NO: 14

SEQ ID NO: 35 - protein, 47 aa, Hepatitis B virus; identical to SEQ ID NO: 15

SEQ ID NO: 36 - protein, 47 aa, Hepatitis B virus; identical to SEQ ID NO: 16

SEQ ID NO: 37 - protein, 47 aa, Hepatitis B virus; identical to SEQ ID NO: 17

SEQ ID NO: 38 - protein, 47 aa, Hepatitis B virus; identical to SEQ ID NO: 18

SEQ ID NO: 39 - protein, 47 aa, Hepatitis B virus; identical to SEQ ID NO: 19

SEQ ID NO: 40 - protein, 47 aa, Hepatitis B virus; identical to SEQ ID NO: 20

SEQ ID NO: 41 - DNA, 3221 bp, Hepatitis B virus
ttccactgccttccaccaagctctgcaggatcccaaagtcaggggtctgtattttcctgctggtggctccagttcaggaacagtcaaccctgctccaaatattgcctctcacatctcgtcaatctccgcgaggactggggaccctgtgccgaacatggagaacatcacatcaggattcctaggacccctgctcgtgttacaggcggggtttttcttgttgacaagaatcctcacaataccgcagagtctagactcgtggtggacttctctcaattttctagggggatcacccgtgtgtcttggccaaaattcgcagtccccaacctccaatcactcaccaacctcctgtcctccaatttgtcctggttatcgctggatgtgtctgcggcgttttatcatattcctcttcatcctgctgctatgcctcatcttcttattggttcttctggattatcaaggtatgttgcccgtttgtcctctaattccaggatcaacaacaaccagtacgggaccatgcaaaacctgcacgactcctgctcaaggcaactctatgtttccctcatgttgctgtacaaaacctatggatggaaattgcacctgtattcccatcccatcgtcctgggctttcgcaaaatacctatgggagtgggcctcagtccgtttctcttggctcagtttactagtgccatttgttcagtggttcgtagggctttcccccactgtttggctttcagctatatggatgatgtggtattgggggccaagtctgtacagcatcgtgagtccctttataccgctgttaccaattttcttttgtctctgggtatacatttaaaccctaacaaaacaaaaagatggggttattccctaaacttcatggtctacataattggaagttggggaacgttgccacaggatcatattgtacaaaagatcaaacactgttttagaaaacttcctgttaacagacctattgattggaaagtatgtcaaagaattgtgggtcttttgggctttgctgctccatttactcaatgtggatatcctgccttaatgcctttgtatgcatgtatacaagctaaacaggcttttactttctcgccaacttacaaggcctttctaagtaaacagtatatgaacctttaccccgttgctcggcaacggcctggtctgtgccaagtgtttgctgacgcaacccccactggctggggcttggccataggccatcagcgcatgcgtggaacctttgtggctcctctgccgatccatactgcggaactcctagccgcttgttttgctcgcagccggtctggagcaaagctcatcggaactgataattctgtcgtcctctcgcggaaatatacatcgtttccatggctgctaggctgtactgccaactggatccttcgcgggacgtcctttgtttacgtcccgtcggcgctgaatcccgcggacgacccctcgcggggccgcttgggagtctctcgtccccttctccgtctgccgttccagccgaccacggggcgcacctctctttacgcggtctccccgtctgtgccttctcatctgccggtccgtgtgcacttcgcttcacctctgcacgttgcatggagaccaccgtgaacgcccatcagatcctgcccaaggtcttacataagaggactcttggactctcagcaatgtcaatgaccgaccttgaggcctacttcaaagactgtgtgtttaaggactgggaggagcttggggaggagattaggttaaaggtgtttgtattaggaggctgtaggcataaattggtctgcgcaccagcaccatgcaactttttcacctctgcctaatcatctcttgtacatgtcccacttttcaagcctccaagctgtgccttgggtggctttggggcatggacattgacccttataaagaatttggagctactgtggagttactctcgtttttgccttctgacttctttccttccgtcagagatctcctagacaccgcctcagctctgtatcgagaagccttagagtctcctgagcattgctctcctcaccatactgcactcaggcaagccattctctgctgggtggaattgatgactctagccacctgggtgggtaataatttggaagatccagcatccagggatctagtagtcaattatgttaatactaacatgggtttaaagatcaggcaactattgtggtttcatatatcttgtcttacttttggaagacagactgtgctagaatatttggtctctttcggagtgtggattcgcactcctccagcttatagaccaccaaatgcccctatcttatcaacacttccggagactactgttgttagacgacgggaccgaggcaggtcccctagaagaagaactccctcgcctcgcagacgcagatctcaatcgccgcgtcgcagaagatctcaatctcgggaatctcaatgttagtattccttggactcataaggtgggaaattttactgggctttattcctctacagtacctatctttaatcctgaatggcaaactccttcctttcctaagattcatttacaagaggacattattaataggtgtcaacaatttgtgggccctctcactgtaaatgaaaagagaagactgaaattaattatgcctgccagattctatcctacccacactaaatatttgcccttagacaaaggaattaaaccttattatccagatcaggtagttaatcattacttccaaaccagacattatttacatactctttggaaggctgggattctatataagagggaaaccacacgtagcgcatcattttgcgggtcaccatattcttgggaacaagagctacatcatgggaggttggtcatcaaaacctcgcaaaggcatggggacgaacctttctgttcccaaccctctgggattctttcccgatcatcagttggaccctgcattcggagccaattcaaacaatccagattgggacttcaaccccatcaaggaccactggccagcaggcaaccaggtaggagtgggagcattcgggccaaggctcacccctccacacggcggtattttggggtggagccctcaggctcagggcatattggccacagtgtcaacaattcctcctcctgcctccaccaatcggcagtcaggaaggcagcctactcccatctctccacctctaagagacagtcatcctgaggccatgcagtggaa

SEQ ID NO: 42 - DNA, 3215 bp, Hepatitis B virus
aactccaccactttccaccaaactcttcaagatcccagagtcagggccctgtaccttcctgctggtggctccagttcagaaatagtgagccctgctcagaatactgtctctgccatatcgtcaatcttatcgaagactggggaccctgtaccgaacatggagaacatcgcatcaggactcctaggacccctgctcgtgttacaggcggggtttttcttgttgacaaaaatcctcacaataccacagagtctagactcgtggtggacttctctcaattttctagggggaacacccgtgtgtcttggccaaaattcgcagtcccaaatctccagtcactcaccaacctgttgtcctccaatttgtcctgggtatcgctggatgtgtctgcggcgttttatcatattcctctgcatcctgctgctatgcctcatcttcttgttggttcttctggactatcaaggtatgttgcccgtttgtcctctaattccaggatcatcaacaaccagcaccggaccatgcaaaacctgcacaactcctgctcaaggaacctctatgtttccctcatgttgctgtacaaaacctacggacggaaactgcacctgtattcccatcccatcatcttgggctttcgcaaaattcctatgggagtgggcctcagtccgtttctcttggctcagtttactagtgccatttgttcagtggttcgtagggctttcccccactgtctggctttcagttatatcgatgatgtggttttgggggccaagtctgtacaacatcttgagtccctttataccgctgttaccaattttcttttgtctttgggtatacatttaaaccctcacaaaacaaaaagatggggatattcccttaacttcatgggatatgtaattgggagttggggcacattgccacaggaacatattgtacaaaaaatcaaaatgtgttttaagaaacttcctgtaaacaggcctattgattggaaagtatgtcaacgaattgtgggtcttttggggtttgccgccccttttacgcaatgtggatatcctgctttaatgcctttatatgcatgtatacaagcaaaacaggcttttactttctcgccaacttacaaggcctttctaagtaaacagtatatgaacctttaccccgttgctcggcaacggcctggtctgtgccaagtgtttgctgacgcaacccccactggttggggcttggccattggccatcagcgcatgcgtgggacctttgtgtctcctctgccgatccatactgcggaactcctagccgcttgttttgctcgcagcaggtctggggcaaaactcatcgggactgacaattctgtcgtgctctcccgcaagtatacatcatttccatggctgctaggctgtgctgccaactggatcctgcgcgggacgtcctttgtttacgtcccgtcggcgctgaatcccgcggacgacccctcccggggccgcttggggctctaccgcccgcttctccgcctgttgtaccgaccgaccacggggcgcacctctctttacgcggactccccgtctgtgccttctcatctgccggaccgtgtgcacttcgcttcacctctgcacgtcgcatggagaccaccgtgaacgcccacaggaacctgcccaaggtcttgcataagaggactcttggactttcagcaatgtcaacgaccgaccttgaggcatacttcaaagactgtgtgtttactgagtgggaggagttgggggaggagattaggttaaaggtctttgtactaggaggctgtaggcataaattggtgtgttcaccagcaccatgcaactttttcacctctgcctaatcatctcatgttcatgtcctactgttcaagcctccaagctgtgccttgggtggctttggggcatggacattgacccgtataaagaatttggagcttctgcggagttactctcttttttaccttctgacttctttccttctattcgagatcttctcgacaccgcctctgctctgtatcgggaggccttagagtctccggaacattgttcacctcaccatacggcactcaggcaagctattctgtgttggggtgagttgatgaatctagccacctgggtgggaagtaatttggaagatccagcatccagggaattagtagtcggctatgtcaacgttaatatgggcctaaaacttagacaactattgtggtttcacatttcctgtcttacttttgggagagaaactgttcttgaatatttggtgtcttttggagtgtggattcgcactccttctgcatatagaccaccaaatgcccctatcctatcaacacttccggaaactactgttgttagacgaagaggcaggtcccctagaagaagaactccctcgcctcgcagacgaaggtctcaatcgccgcgtcgcagaagatctcaatctcgggaatctcaatgttagtattccttggacacataaggtgggaaactttacggggctttattcttctacggtaccttgttttaatcctaaatggcaaactccttcttttcctgacattcatttgcaggaggacattgttgatagatgtaagcaatttgtggggccccttacagtaaatgaaaacaggagactaaaattaattatgcctgctaggttttatcccaatgttactaaatatttgcccttagataaagggatcaaaccgtattatccagagtatgtagttaatcattacttccagacgcgacattatttacacactctttggaaagcggggatcttatataaaagagagtccactcgtagcgcctcattttgcgggtcaccatattcttgggaacaagatctacagcatgggaggttggtcttccaaacctcgaaaaggcatggggacaaatctttctgtccccaatcccctgggattcttccccgatcatcagttggaccctgcattcaaagccaactcagaaaatccagattgggacctcaacccgcacaaggacaactggccggacgccaacaaggtgggagtgggagcattcgggccagggttcacccctccccatggggggctgttggggtggagccctcaggctcagggcctactcacaactgtgccagcagctcctcctcctgcctccaccaatcggcagtcaggaaggcagcctactcccttatctccacctctaagggacactcatcctcaggccatgaagtgg

SEQ ID NO: 43 - DNA, 3215 bp, Hepatitis B virus
aattccacaacattccaccaagctctgctagaccccagagtgaggggcctatactttcctgctggtggctccagttccggaacagtaaaccctgttccgactactgcctcacccatatcgtcaatcttctcgaggactggggaccctgcaccgaacatggagagcacaacatcaggattcctaggacccctgctcgtgttacaggcggggtttttcttgttgacaagaatcctcacaataccacagagtctagactcgtggtggacttctctcaattttctagggggagcacccacgtgtcctggccaaaattcgcagtccccaacctccaatcactcaccaacctcttgtcctccaatttgtcctggctatcgctggatgtgtctgcggcgttttatcatattcctcttcatcctgctgctatgcctcatcttcttgttggttcttctggactaccaaggtatgttgcccgtttgtcctctacttccaggaacatcaactaccagcacgggaccatgcaagacctgcacgagtcctgctcaaggaacctctatgtttccctcttgttgctgtacaaaaccttcggacggaaactgcacttgtattcccatcccatcatcctgggctttcgcaagattcctatgggagtgggcctcagtccgtttctcctggctcagtttactagtgccatttgttcagtggttcgtagggctttcccccactgtttggctttcagttatatggatgatgtggtattgggggccatgtctgtacaacatcttgagtccctttttacctctattaccaattttcttttgtctttgggtatacatttgaaccctaataaaaccaaacgttggggctactcccttaacttcatgggatatgtaattggaagttggggtactttaccgcaagaacatattgtacaaaaacttaagcaatgttttcgaaaactgcctgtaaatagacctattgattggaaagtatgtcagagaattgtgggtcttttgggctttgctgccccttttacacaatgtggctatcctgctttaatgcctttatatgcatgtatacaatctaagcaggctttcactttctcgccaacttacaaggcctttctgtgtaaacaatatctgaacctttaccccgttgcccggcaacggtcaggtctctgccaagtgtttgctgacgcaacccccactggatggggcttggctattggccatcgccgcatgcgtggaacctttgtggctcctctgccgatccatactgcggaactcctagcagcttgttttgctcgcagccggtctggagcaaaacttatcggcaccgacaactctgttgtcctctctcggaagtacacctcctttccatggctgctagggtgtgctgccaactggatcctgcgcgggacgtcctttgtttacgtcccgtcggcgctgaatcccgcggacgacccgtctcggggccgtttgggactctaccgtccccttcttcatctgccgttccggccgaccacggggcgcacctctctttacgcggtctccccgtctgtgccttctcatctgccggaccgtgtgcacttcgcttcacctctgcacgtcgcatggagaccaccgtgaacgcccaccaggtcttgcccaaggtcttacataagaggactcttggactctcagcaatgtcaacgaccgaccttgaggcatacttcaaagactgtttgtttaaggactgggaggagttgggggaggagattaggttaaaggtctttgtactaggaggctgtaggcataaattggtctgttcaccagcaccatgcaactttttcacctctgcctaatcatctcatgttcatgtcctactgttcaagcctccaagctgtgccttgggtggctttggggcatggacattgacccgtataaagaatttggagcttctgtggagttactctcttttttgccttctgacttctttccttctattcgagatctcctcgacaccgcctctgctctgtatcgggaggccttagagtctccggaacattgttcgcctcaccatacagcactcaggcaagctattctttgttggggtgagttgatgaatctggccacctgggtgggaagtaatttggaagacccagcatccagggaattagtagccagctatgtcaatgttaatatgggcctaaaaatcagacaactactgtggtttcacatttcctgtcttacttttggaagagaaactgttcttgagtatttggtatcttttggagtgtggattcgcactcctcctgcttacagaccaccaaatgcccctatcttatcaacacttccggaaactactgttgttagacgacgaggcaggtcccctagaagacgaactccctcgcctcgcagacgaaggtctcaatcgccgcgtcgcagaagatctcaatctcgggaatctcaatgttagtatcccttggactcataaggtgggaaactttactgggctttattcttctactgtacctgtctttaatccagagtggcaaactccctcctttcctcacattcatttacaggaggacattattaatagatgtcaacaatatgtgggccctcttacagttaatgaaaaaagaagattaaaattaattatgcctgctaggttctatcctaaccttaccaaatatttgcccttggacaaaggcattaaaccatattatcctgaacatgcagttaatcattacttcaaaactaggcattatttacatactctgtggaaggctggcattctatataagagagaaactacacgcagcgcctcattttgtgggtcaccatattcttgggaacaagagctacagcatgggaggttggtcttccaaacctcgacaaggcatggggacaaatctttctgttcccaatcctctgggattctttcccgatcaccagttggaccctgcgttcggagccaactcaaacaatccagattgggacttcaaccccaacaaggatcactggccagaggcaaatcaggtaggagcgggagcattcgggccagggttcaccccaccacacggcggtcttttggggtggagccctcaggctcagggcatactgacaacagtgccagtagcacctcctcctgcctccaccaatcggcagtcaggaagacagcctactcccatctctccacctctaagagacagtcatcctcaggccatgcagtgg

SEQ ID NO: 44 - DNA, 3182 bp, Hepatitis B virus
aactccacaaccttccaccaaactctgcaagatcccagagtgagaggcctgtatttccctgctggtggctccagttcaggaacagtaaaccctgttccgactactgtctctcccatatcgtcaatcttctcgaggattggggaccctgcgctgaacatggagaacatcacatcaggattcctaggacccctgctcgtgttacaggcggggtttttcttgttgacaagaatcctcacaataccgcagagtctagactcgtggtggacttctctcaattttctagggggaactaccgtgtgtcttggccaaaattcgcagtccccaacctccaatcactcaccaacctcctgtcctccaacttgtcctggttatcgctggatgtgtctgcggcgttttatcatcttcctcttcatcctgctgctatgcctcatcttcttgttggttcttctggactatcaaggtatgttgcccgtttgtcctctaattccaggatcttcaactaccagcacgggaccatgcagaacctgcacgactcctgctcaaggaacctctatgtatccctcctgttgctgtaccaaaccttcggacggaaattgcacctgtattcccatcccatcatcctgggctttcggaaaattcctatgggagtgggcctcagcccgtttctcctggctcagtttactagtgccatttgttcagtggttcgtcgggctttcccccactgtttggctttcagttatatggatgatgtggtattgggggccaagtctgtacagcatcttgagtccctttttaccgctgttaccaattttcttttgtctttgggtatacatttaaaccctgacaaaacaaaaagatggggttactctttacatttcatgggctatgtcattggaagttatgggtcattgccacaagatcacatcatacaaaaaatcaaagaatgttttcgaaaacttcctgttaacagacctattgattggaaagtctgtcaacgtattgtgggtcttttgggttttgctgccccttttacacaatgtggttatcctgctttaaagcctttgtatgcatgtattcaatctaagcaggctttcactttctcgccaacttacaaggcctttctgtgtaaacaatacctgaacctttaccccgttgcccggcaacggccaggtctgtgccaagtgtttgctgacgcaacccccactggctggggcttggtcatgggccatcagcgcatgcgtggaacctttctggctcctctgccgatccatactgcggaactcctagccgcttgttttgctcgcagcaggtctggagcaaacattctcgggacggataactctgttgttctctcccgcaaatatacatcgtttccatggctgctaggctgtgctgccaactggatcctgcgcgggacgtcctttgtttacgtcccgtcggcgctgaatcccgcggacgacccttctcggggtcgcttgggactctctcgtccccttctccgtctgccgtttcgaccgaccacggggcgcacctctctttacgcggactccccgtctgtgccttctcatctgccggaccgtgtgcacttcgcttcacctctgcccgtcgcatggagaccaccgtgaacgcccaccgagtcttgcccaaggtcttacataagaggactcttggactctctgtaatgtcaacgaccgaccttgaggcatacttcaaagactgtttgttcaaagactgggaggagttgggggaggagattagattaaaggtctttgtactaggaggctgtaggcataaattggtctgcgcaccagcaccatgcaactttttcacctctgcctaatcatctcttgttcatgtcctactgttcaagcctccaagctgtgccttgggtggctttagggcatggacatcgatccttataaagaatttggagctactgtggagttactctcgtttttgccttctgacttctttccttcagtacgagatcttctagataccgcctcagctctgtatcgggaagccttagagtctcctgagcattgttcacctcaccatactgcactcaggcaagcagttctgtgctggggggaactaatgactctagctacctgggtgggtggtaatttggaagatccaacatccagggacctagtagtcagttatgtcaacactaatatgggcctaaagttccggcaactattgtggtttcacatttcttgtctcacttttggaagagaaacagttttagagtatttggtgtctttcggagtgtggattcgcactcctccagcttatagaccaccaaatgcccctatcttatcaacacttccggagactactgttgttagacgacgaggcaggtcccctagaagaagaactccctcgcctcgcagacgaaggtctcaatcgccgcgtcgcagaagatctcaatctcgggaatctcaatgttagtattccttggactcataaggtgggaaactttacggggctttattcttctactgtacctgtctttaaccctcattggaaaacaccctcttttcctaatatacatttacaccaagacattatcaaaaaatgtgaacaatttgtaggcccactcacagtcaatgaaaaaagaagactgcaattgattatgcctgctaggttttatccaaatgttaccaaatatttgccattggataagggtatcaaaccttattacccagaacatctagttaatcattacttccaaaccagacattatttacacactctatggaaggcgggtatattatataagagagaaacaacacatagcgcctcattttgtgggtcaccatattcttgggaacaaaagctacagcatggggcagaatctttccaccagcaatcctctgggattctttcccgaccaccagttggatccagccttcagagcaaacaccgcaaatccagattgggacttcaatcccaacaaggacacctggccagacgccaacaaggtaggagctggagcattcgggctgggattcaccccaccgcacggaggccttttggggtggagccctcaggctcagggcatactacaaaccttgccagcaaatccgcctcctgcctctacccatcgccagtcaggaaggcagcctaccccgctgtctccacctttgagaaacactcatcctcaggccatgcagtgg

SEQ ID NO: 45 - DNA, 3212 bp, Hepatitis B virus
ttccacagcattccaccaagctctgcaggatcccaaagtaagaggcctgtattttcctgctggtggctccagttccggaacagtgagccctgttccgactactgcctcactcatctcgtcaatcttctcgaggattggggaccctgcaccgaacatggaaggcatcacatcaggattcctgggacccctgctcgtgttacaggcggggtttttcttgttgacaaaaatcctcacaataccgcagagtctagactcgtggtggacttctctcaattttctagggggagctcccgtgtgtcttggccaaaattcgcagtccccaacctccaatcactcaccaacctcttgtcctccgatttgtcctggctatcgctggatgtgtctgcggcgttttatcatcttcctcttcatcctgctgctatgcctcatcttcttgttggttcttctggactatcaaggtatgttgcccgtttgtcctctaattccaggatcatcaaccaccagtacgggaccctgccgaacctgcacgactcttgctcaaggaacctctatgtttccctcatgttgctgttcaaaaccttcggacggaaattgcacttgtattcccatcccatcatcatgggctttcggaaaattcctatgggagtgggcctcagcccgtttctcctggctcagtttactagtgccatttgttcagtggttcgccgggctttcccccactgtctggctttcagttatatggatgatgtggtattgggggccaagtctgtacaacatcttgagtccctttatacctctgttaccaattttcttttgtctttgggtatacatttaaatcccaacaaaacaaaacgatggggatattctcttaatttcatgggatatgtaattgggagttgggggtcattaccacaggaacacatccgaatgaaaatcaaagactgttttagaaaactccctgttaaccggcctattgattggaaagtatgtcaaagaattgtgggtcttttgggctttgctgccccttttacacaatgtggatatcctgctttaatgcctctgtatgcgtgtgttcaatcgaagcaggctttcactttctcgccaacttacaaggcctttctgtgtaaacaatacctgaacctttaccccgttgcccggcaacggccaggtctgtgccaagtgtttgctgatgcaacccccactggctggggcttggccataggccatcagcgcatgcgtggaacctttgtggctcctctgccgatccatactgcggaactcctagccgcttgttttgctcgcagcaggtctggagcgaaacttatcgggacggataattctgtcgttctctcccggaaatatacatcatttccatggctgctaggctgtgctgccaactggatcctgcgagggacgtcctttgtctacgtcccgtcagcgctgaatcctgcggacgacccgtctcggggtcgcttggggatctatcgtccccttctccgtctgccgttccggccgaccacggggcgcacctctctttacgcggtctccccgtctgtgccttctcatctgccggaccgtgtgcacttcgcttcacctctgcacgtcgcatggagaccaccgtgaacgcccatcaaatcttgcccaaggtcttacataagcggactcttggactttctgcaatgtcaacgaccgaccttgaggcatacttcaaagactgtttgtttaaagactgggaggagttgggggaggagattagattaaaggtctttgtactaggaggctgtaggcataaattggtctgcgcaccagcaccatgcaactttttcacctctgcctaatcatctcttgttcatgtcctactgttcaagcctccaagctgtgccttgggtggctttggggcatggacattgacccttataaagaatttggagctactgtggagttactctcgtttttgccgtctgacttctttccgtcagttagagatcttctagataccgcctcagctctgtatcgggatgccttagaatctcctgagcattgttcacctcaccatactgcactcaggcaagccattctttgctggggggaactaatgactctagctacctgggtgggtgtaaatttggaagatccagcatccagggacctagtagtcagttatgtcaatactaatatgggcctaaagttcaggcaattattgtggtttcacatttcttgtctcacttttggaagagaaaccgtcatagagtatttggtgtcttttggagtgtggattcgcactcctccagcttatagaccaccaaatgcccctatcttatcaacacttccggagaatactgttgttagacgaagaggcaggtcccctagaagaagaactccctcgcctcgcagacgaagatctcaatcgccgcgtcgcagaagatctcaatctccagcttcccaatgttagtattccttggactcacaaggtgggaaattttacgggcctttactcttctactatacctgtctttaatcctaactggaaaactccatcttttcctgatattcatttgcaccaagacattattaacaaatgtgaacaatttgtaggtcctctaacagtaaatgaaaaacgaagattaaacttagtcatgcctgctagattttttcccatctctacgaaatatttgcccctagagaagggtataaaaccttattatccagataatgtagttaatcattacttccaaaccagacactatttacataccctatggaaggcgggcatcttatataaacgggaaactacacgtagcgcctcattttgtgggtcaccttattcttgggaacaagagctacatcatggggctttcttggacggtccctctcgaatgggggaagaatcattccaccaccaatcctctgggattttttcccgaccaccagttggatccagcattcagagcaaacaccagaaatccagattgggaccacaatcccgacaaagaccactggacagaagccaacaaggtaggagtgggagcattcgggccggggttcactcccccacacggaggccttttggggtggagccctcaggctcaaggcatgctaaaaacattgccagcagatccgcctcctgcctccaccaatcggcagtcaggaaggcagcctaccccaatcactccacctttgagagacactcatcctcaggccatgcagtggaa

SEQ ID NO: 46 - DNA, 3215 bp, Hepatitis B virus
ctccactcagttccaccaggctctgttagatccgagagtaagggctctgtattttcctgctggtggctccagttcagagacacagaaccctgctccgactattgcctctctcacatcatcaatcttcttgaagactgggggccctgctacgaacatggacaacatcacatcaggactcctaggacccctgctcgtgttacaggcggtgtgtttcttgttgacaaaaatcctcacaataccacagagtctagactcgtggtggacttctctcaattttctagggggaacacccgggtgtcctggccaaaattcgcagtccccaacctccaatcacttaccaacctcctgtcctccaacttgtcctggctatcgctggatgtgtctgcggcgttttatcatcttcctcttcatcctgctgctatgcctcatcttcttgttggttcttctggactatcaaggtatgttgcccgtttgtcctctacttccaggatccacgaccaccagcacgggaccatgcaaaacctgcacaactcttgctcaaggaacctctatgtttccctcttgctgctgttccaaaccctcggacggaaactgcacttgtattcccatcccatcatcctgggctttaggaaaatacctatgggagtgggcctcagcccgtttctcctggctcagtttactagtgcaatttgttcagtggtgcgtagggctttcccccactgtctggcttttagttatatggatgatctggtattgggggccaaatctgtgcagcatcttgagtccctttataccgctgttaccaattttctgttatctgtgggtatccatttaaatacctcgaaaacaaaaagatggggttataccctaaatttcatgggttatgttattggcagttggggatcattaccacaagatcacattgtacaaaaaatcaaagattgttttcgtaaacttcctgtaaatcgccctattgattggaaagtttgtcaacgcattgtgggtcttttgggctttgccgccccctttactcaatgtggttatcctgctctcatgcctctgtatgcctgtataactgctaaacaggcttttgtcttttcgccaacttacaaggcctttctatgtcaacaatacatgaacctttaccccgttgctcggcaacggccaggcctgtgccaagtgtttgctgacgcaacccccactggttggggcttggccattggccatcagcgcatgcgtggaacctttgtggctcctctgccgatccatactgcggaactccttgcagcttgtttcgctcgcagccggtctggagcgaaactcatcggcacagacaactctgttgtcctctctaggaagtacacctccttcccatggctgctcggttgtgctgccaactggatcctacgcgggacgtcctttgtttacgtcccgtcggcgctgaatccagcggacgatccctctcggggtcgcttggggctgtatcgcccccttctccgtctgccgttccagccgacgacgggtcgcacctctctttacgcggcctccccgtctgttccttctcgtctgccggaccgtgtgcacttcgcttcacctctgcacgtcgcatggagaccaccgtgaacgcccctcgaagcttgccaacagtcttacataagcggactcttggactttcaggaaggtcaatcacctggatcgaagaatacatcaaagactgtgtatttaaggactgggaggagctgggggaggagattaggttaaaggtctttgtattaggaggctgtaggcataaattggtctgttcaccagcaccatgcaactttttcacctctgcctaatcatcttttgttcatgtcctactgttcaagcctccaagctgtgccttgggtggctttggggcatggacattgacccttataaagaatttggagcttctgtggaattactctcttttttgccttctgacttcttcccgtcagttcgggacctactcgacaccgcttcagccctctaccgggatgctttagaatcaccagaacattgcacacctaaccataccgctctcaggcaagctatattgtgctggggtgagttaatgactttggcttcctgggtgggcaataacttggaagatcctgctgctagggacctagtggttaactatgtcaatactaacatgggcctaaaaattagacaattgctgtggtttcacatttcctgccttacttttggaagagaaacagttcttgagtatttggtgtcttttggagtgtggattcgcactcctcctgcttatagaccaccaaatgcccctatcttatccacacttccggaaactactgttgttagacgacgaggcaggtcccctcgaagaagaactccctcgcctcgcagacgaaggtctcaatcgccgcgtcgcagaagatctcaatctccagcttcccaatgttagtattccttggactcataaggtgggaaattttacgggactctattcctctactgttcctacttttaatcctgactggttaactccttcttttcctgacattcatttacatcaagatttgatacacaaatgtgaacaatttgtaggccctctcacaaaaaatgaattgagaagattaaaattagttatgccatccagattttttcctaaggttaccaaatattttcctatggaaaagggaattaaaccctattatcctgataacgtggttaatcattattttaagaccagacactatttgcatactttatggaargcrggcattctatataagagagaatccacacgtagcgcctcattttgtgggtcaccatattcttgggaacaagagctacagcatgggagcacctctatcaacgactcgaaggggcatgggacagaatctctctgtacccaatcctctgggattctttccagaccatcagctggatcctctattcagggcaaattccagcagtcccgactgggacttcaacaaaaacaaggacaattggccaatggcaaacaaggtaggagtgggaggatacggtcctgggttcacacccccacacggtggcctgttggggtggagtccacaggcacagggtgtgcttacaacattgccagcagatccgcctcctgcttccaccaatcggcggtccgggagaaaaccaaccccagtctctccacctctaagagacactcatccacaggccatgcagtggaa

SEQ ID NO: 47 - DNA, 3248 bp, Hepatitis B virus
ctctacagcattccaccaagctctacaaaatcccaaagtcaggggcctgtattttcctgctggtggctccagttcagggatagtgaaccctgttccgactattgcctctcacatctcgtcaatcttctccaggattggggaccctgcaccgaacatggagaacatcacatcaggattcctaggacccctgctcgtgttacaggcggggtttttcttgttgacaagaatcctcacaataccgcagagtctagactcgtggtggacttctctcaattttctagggggagtgcccgtgtgtcctggcctaaattcgcagtccccaacctccaatcactcaccaatctcctgtcctccaacttgtcctggctatcgctggatgtgtctgcggcgttttatcatattcctcttcatcctgctgctatgcctcatcttcttgttggttcttctggactatcaaggtatgttgcccgtttgtcctctgattccaggatcctcgaccaccagcacgggaccctgcaaaacctgcacgactcctgctcaaggcaactctatgtatccctcatgttgctgtacaaaaccttcggacggaaattgcacctgtattcccatcccatcatcttgggctttcgcaaaatacctatgggagtgggcctcagtccgtttctcttggctcagtttactagtgccatttgttcagtggttcgtagggctttcccccactgtctggctttcagctatatggatgatgtggtattgggggccaaatctgtacaacatcttgagtccctttataccgctgttaccaattttcttttgtctttgggtatacatctaaaccctaacaaaacaaaaagatggggttattccttaaattttatgggatatgtaattggaagttggggtactttgccacaagaacacatcacacagaaaattaagcaatgttttcggaaactccctgttaacaggccaattgattggaaagtctgtcaacgaataactggtctgttgggtttcgctgctccttttacccaatgtggttaccctgccttaatgcctttatatgcatgtatacaagctaagcaggcttttactttctcgccaacttataaggcctttctctgtaaacaatacatgaacctttaccccgttgctaggcaacggcccggtctgtgccaagtgtttgctgacgcaacccccactggttggggcttggccatcggccatcagcgcatgcgtggaacctttgtggctcctctgccgatccatactgcggaactcctagctgcttgttttgctcgcagccggtctggagcaaaactcattgggactgacaattctgtcgtcctttctcggaaatatacatcctttccatggctgctaggctgtgctgccaactggatccttcgcgggacgtcctttgtttacgtcccgtcagcgctgaatccagcggacgacccctcccggggccgtttggggctctgtcgcccccttctccgtctgccgttcctgccgaccacggggcgcacctctctttacgcggtctccccgtctgttccttctcatctgccggaccgtgtgcacttcgcttcacctctgcacgttacatggaaaccgccatgaacacctctcatcatctaccaaggcagttatataagaggactcttggactgtttgttatgtcaacaaccgggatggagaaatacttcaaggactgtgtttttgctgagtgggaagaattaggcaatgagtccaggttaatgacctttgtattaggaggctgtaggcataaattggtctgcgcaccagcaccatgtaactttttcacctctgcctaatcatctcttgttcatgtcctactgttcaagcctccaagctgtgccttgggtggctttagggcatggatagaacaactttgccatatggcctttttggcttagacattgacccttataaagaatttggagctactgtggagttgctctcgtttttgccttctgactttttcccgtctgttcgtgatcttctcgacaccgcttcagctttgtaccgggaatccttagagtcctctgatcattgttcgcctcaccatacagcactcaggcaagcaattctgtgctggggtgagttgatgactctagctacctgggtgggtaataatttggaagatccagcatccagagatttggtggtcaattatgttaatactaatatgggtttaaaaatcaggcaactattgtggtttcacatttcctgtcttacttttgggagagaaaccgttcttgagtatttggtgtcttttggagtgtggattcgcactcctcctgcttatagaccaccaaatgcccctatcctatcaacacttccggagactactgttgttagacgaagaggcaggtcccctcgaagaagaactccctcgcctcgcagacgaagatctcaatcgccgcgtcgcagaagatctgcatctccagcttcccaatgttagtattccttggactcacaaggtgggaaactttacggggctgtattcttctactatacctgtctttaatcctgattggcaaactccttcttttccaaatatccatttgcatcaagacattataactaaatgtgaacaatttgtgggccctctcacagtaaatgagaaacgaagattaaaactagttatgcctgccagatttttcccaaactctactaaatatttaccattagacaaaggtatcaaaccgtattatccagaaaatgtagttaatcattacttccagaccagacattatttacataccctttggaaggcgggtattctatataagagagaaacatcccgtagcgcttcattttgtgggtcaccatatacttgggaacaagatctacagcatggggctttcttggacggtccctctcgagtggggaaagaacctttccaccagcaatcctctaggattccttcccgatcaccagttggacccagcattcagagcaaataccaacaatccagattgggacttcaatcccaaaaaggacccttggccagaggccaacaaggtaggagttggagcctatggacccgggttcacccctccacacggaggccttttggggtggagccttcagtctcagggcacactaacaactttgccagcagatccgcctcctgcctccaccaatcgtcagtcagggaggcagcctactcccatctctccaccactaagagacagtcatcctcaggccatgcagtggaa

SEQ ID NO: 48 - DNA, 3215 bp, Hepatitis B virus
ctcaacacagttccaccaagcactgttggatccgagagtaagggggctgtattttcctgctggtggctccagttcagaaacacagaaccctgctccgactattgcctctctcacatcatcaatcttctcgaagactggggaccctgctatgaacatggagaacatcacatcaggactcctaggaccccttctcgtgttacaggcggtgtgtttcttgttgacaaaaatcctcacaataccaaagagtctagactcgtggtggacttctctcaattttctaggggtaccacccgggtgtcctggccaaaattcgcagtccccaatctccaatcacttaccaacctcctgtcctccaacttgtcctggctatcgttggatgtgtctgcggcgttttatcatcttcctcttcatcctgctgctatgcctcatcttcttgttggttcttctggactatcaaggtatgttgcccgtgtgtcctctacttccaggatcwacaaccaccagcacgggaccctgcaaaacctgcaccactcttgctcaaggaacctctatgtttccctcctgctgctgtaccaaaccttcggacggaaattgcacctgtattcccatcccatcatcttgggctttcggaaaatacctatgggagtgggcctcagcccgtttctcttggctcagtttactagtgcaatttgttcagtggtgcgtagggctttcccccactgtctggcttttagttatatggatgatctggtattgggggccaaatctgtgcagcatcttgagtccctttataccgctgttaccaattttttgttatctgtgggcatccatttgaacacagctaaaacaaaatggtggggttattcccttcactttatgggttatataattgggagttgggggaccttgcctcaggaacatattgtgcataaaatcaaagattgctttcgcaaacttcccgtgaatagacccattgattggaaggtttgtcaacgcattgtgggtcttttgggctttgcagccccttttactcaatgtggttatcctgctctcatgcccttgtatgcctgtattrccgctaagcaggcttttgttttctcgccaacttacaaggcctttctctgtaaacaatacatgaacctttaccccgttgctcggcaacggccaggcctttgccaagtgtttgctgacgcaacccccactggctggggcttggcgattggccatcagcgcatgcgcggaacctttgtggctcctctgcccatccatactgcggaactcctagccgcttgtttcgctcgcagcaggtctggagcggacattatcggcactgacaactccgttgtcctttctcggaagtacacctccttcccatggctgctaggctgtgctgccaactggatcctgcgcgggacgtcctttgtctacgtcccgtcggcgctgaatcctgcggacgacccctctcgtggtcgcttggggctctgccgccctcttctccgcctgccgttccggccgacgacgggtcgcacctctctttacgcggactccccgcctgtgccttctcatctgccggcccgtgtgcacttcgcttcacctctgcacgtcgcatggagaccaccgtgaacgccccttggaacttgccaacaaccttacataagaggactcttggactttcgccccggtcaacgacctggattgaggaatacatcaaagactgtgtatttaaggactgggaggagtcgggggaggagttgaggttaaaggtctttgtattaggaggctgtaggcataaattggtctgttcaccagcaccatgcaactttttcacctctgcctaatcatcttttgttcatgtcccactgttcaagcctccaagctgtgccttgggtggctttggggcatggacattgacccttataaagaatttggagcttctgtggagttactctcatttttgccttctgacttcttcccgtctgtccgggacctactcgacaccgcttcagccctctaccgagatgccttagaatcaccagaacattgcacccccaaccacactgctctcaggcaagctattttgtgctggggtgagttgatgaccttggcttcctgggtgggcaataatttagaggatcctgcagcaagagatctagtagttaattatgtcaatactaacatgggcctaaaaattagacaattattatggtttcacatttcttgccttacatttggaagagaaactgtgcttgagtatttggtgtcttttggagtgtggattcgcactccacctgcttatagaccaccaaatgcccctatcctatcaacacttccggagactactgttgttagacaacgaggcagggcccctagaagaagaactccctcgcctcgcagacgaagatctcaatctccgcgtcgcagaagatctcaatctccagcttcccaatgttagtattccttggactcataaggtgggaaactttaccggtctttactcctctactatacctgttttcaatcctgactggttaactccttcttttcctgacattcacttgcatcaagatctgatacaaaaatgtgaacaatttgtaggcccactcactacaaatgaaaggagacgattgaaactaattatgccagctaggttttatcccaaagttactaaatacttccctttggataaaggtattaagccttactatccagagaatgtggttaatcattactttaaaactagacattatttacatactttgtggaaggcaggaattctatataagagagaatccacacatagcgcctcattttgtgggtcaccatattcctgggaacaagagctacagcatgggagcacctctctcaacggcgagaaggggcatgggacagaatctttctgtgcccaatcctctgggattctttccagaccaccagttggatccactattcagagcaaattccagcagtcccgattgggacttcaacacaaacaaggacaattggccaatggcaaacaaggtaggagtgggaggcttcggtccagggttcacacccccacacggtggccttctggggtggagccctcaggcacagggcattctaacaacctcgccaccagatccacctcctgcttccaccaatcggaggtcaggaagaaagccaaccccagtctctccacctctaagggacacacatccacaggccatgcagtggaa

SEQ ID NO: 49 - protein, 47 aa, Artificial Sequence
  Description of Artificial Sequence: Synthetic polypeptide
  N-term Myr
  C-term NH2
GLNQSTFNPLGFFPSHQLDPLFKANAGSADWDKNPNKDPWPQAHDTA